European Patent Specification EP 3 235 907 B1, published June 21, 2023. Title: Metabolically engineered organisms for the production of added value bio-products. Applicant: UNIVERSITEIT GENT. The sequence listing filed with the application follows.

SEQUENCE LISTING (54 sequences)

SEQ ID NO: 1 - protein, 768 aa, Dictyostellium discoideum
MNDSPIISVVLPFLIKDNDDKSLNYQGINNLIISIDSIIEQTFKEWELILVDDGSNNEILEQLLSKRYSTDNRIKFIINKENKGIVKSLNDAILNHCSPTSKYIARMDSDDISHPTRLQSQLKYLQSNETIDILGCPIKMFNNNKLIEILNNNNNNNNINNNVKELINIINNEESFKFIQHPDKDILMWSMFFNCCIVHPSVIFKRSIFTIEHCYEENNQFPFIEDYLFWLKSLIMKGLNISNIQSSTPLLYLRKHNNSISFKNIEKQKDSTANASCYYLNILFKRFNIDSEIIQNSSLSMKEIIQFFQLSPSSLSKINNISIELFEFAFKYLELIEKSCTKQQPNYSNSIKDAANEKMGELVSLCLSNYPNNQKSSLLWEKWLSRNPTSQLLSLLSNLNVKSSTTIINNNINNNNNNNNNNNNNNNNNNNNNNNNNNNNSILNFISGINSNKINTPKSNNNKFKENGIRIICFSKDRAFQLKEYLRTFFKYLKNDDNGNDKFEIIVDVLFTYSNEKFKNSYQLVIESFPQVNFIKEENFTDQLINLVQKTNKLEYVMFSVDDILYYNEFNLKEYCLSLNSEPLALGFYMKLNKNITYCHTCNQDITIPLNSNTISRTENNFKYLKWNRNDNDCKKDWNYPWDLCSTIYRCNDIDSIINGIVKYYGIRNGINHPNRFEFNGNRPIIQKQIYQNKPYCLCLSDHYSPMSVVTINRVQDVYDNPIYDQTLSLDDLDQLLYSNKSLNDEKYKENSLSLNFKSVHIGELFIS

SEQ ID NO: 2 - DNA, 2307 bp, Artificial sequence
  codon optimized sequence encoding SEQ ID NO 1
atgaacgatagcccgattattagcgttgttctgccgtttctgatcaaagataacgatgataaaagcctgaactaccagggcattaacaacctgattattagcatcgatagcatcatcgagcagacctttaaagaatgggaactgattctggttgatgatggcagcaataacgaaattctggaacagctgctgagcaaacgttatagcaccgataaccgcatcaaatttattattaataaagaaaataaaggcattgtgaaaagcctgaatgatgccattctgaatcattgtagcccgaccagcaaatatattgcacgtatggatagcgacgatattagccatccgacccgtctgcagagccagctgaaatatctgcagagcaatgaaaccattgatattctgggttgcccgatcaaaatgtttaataataataaactgattgaaattctgaataataataacaataacaacaatattaataataatgtgaaagaactgattaatattattaataatgaagaaagctttaaatttattcagcatccggataaagatattctgatgtggtccatgttcttcaattgctgtattgttcatccgagcgtgatttttaaacgcagcatttttaccatcgagcactgctatgaagagaataatcagtttccgttcatcgaggattacctgttttggctgaaatccctgattatgaaaggcctgaacattagcaatatccagagcagcacaccgctgctgtatctgcgtaaacataataacagcattagctttaaaaatattgaaaaacagaaagatagcaccgccaatgccagctgttattatctgaacattctgttcaaacgctttaacatcgacagcgaaattattcagaatagcagcctgagcatgaaagaaatcatccagttttttcagctgagcccgagcagcctgtccaaaattaataacattagcatcgaactgtttgaatttgcctttaaatatctggaactgatcgagaaaagctgtaccaaacagcagccgaattatagcaacagcattaaagatgcagccaacgaaaaaatgggtgaactggttagcctgtgtctgagcaattatccgaataatcagaaaagcagtctgctgtgggaaaaatggctgagccgtaatccgaccagccagctgctgagtctgctgagcaatctgaatgttaaaagcagcaccaccattattaataacaatattaacaacaacaataataataacaacaataataacaataacaataacaataataacaacaacaacaataataataataacaacaacagcattctgaattttattagcggcattaatagcaataaaattaataccccgaaaagcaacaataacaaatttaaagagaatggcattcgcattatttgcttcagcaaagatcgtgcattccagctgaaagaatatctgcgcaccttcttcaaatatctgaaaaatgatgataatggcaatgataaatttgaaattattgtggatgtgctgtttacctatagcaatgaaaaattcaaaaatagctatcagctggtgatcgaaagctttccgcaggttaactttattaaagaagaaaactttaccgatcagctgattaacctggtgcagaaaaccaacaaactggaatatgtgatgttcagcgtggatgatatcctgtattacaacgagttcaatctgaaagagtattgcctgagcctgaatagcgaaccgctggcactgggtttttatatgaaactgaataaaaatattacctattgccatacctgcaaccaggatattaccattccgctgaatagcaataccattagccgcaccgaaaataactttaaatacctgaaatggaatcgcaacgataatgattgcaaaaaagactggaactatccgtgggatctgtgtagcaccatttatcgttgcaacgacattgacagcatcattaatggtattgtgaaatattatggtattcgcaacggcattaatcatccgaatcgctttgaatttaatggcaaccgtccgattattcagaaacaaatctaccagaacaaaccgtattgtctgtgcctgagcgatcattattcaccgatgagcgttgttaccattaatcgtgttcaggatgtgtatgataacccgatttatgatcagaccctgagcctggatgatctggatcaactgctgtatagcaataaatccctgaacgatgaaaaatataaagaaaacagcctgagtctgaacttcaaaagcgttcatattggcgaactgttcatcagctaa

SEQ ID NO: 3 - DNA, 2307 bp, Dictyostellium discoideum
atgaatgattcaccaataataagtgtagttttaccttttttaataaaggacaatgacgataaatcattaaattaccaaggaataaataatttaataatatcaatagatagcattattgaacaaacttttaaagaatgggaattaattttagttgatgatggatcaaataatgaaattttggagcaattactttcaaaaagatatagtacagataatagaattaaattcataataaataaagagaataaaggtattgttaaaagtttaaatgatgcaattttaaatcattgttcaccaacttcaaaatatattgctcgtatggattcagatgatatttctcatccaacaagattacaatctcaacttaaatatcttcaatcaaatgaaacaattgatatattaggttgtccaattaaaatgtttaataataataaattaattgaaattttaaataataataataataataataatattaataataatgtgaaagagttaattaatataattaataatgaagaatcttttaaatttattcaacatcctgataaagatattttaatgtggtcaatgtttttcaattgttgtattgttcacccttctgtaatatttaaaagatcgatattcactattgaacattgttatgaagaaaacaaccaatttccattcattgaagattacttattttggttaaaatccttaataatgaaaggtttaaatatttcaaatatccaatcatcaacaccattactatatttaagaaaacataataactctatatcttttaaaaatattgaaaaacaaaaagattccactgctaatgcatcttgttattatctaaatatactttttaaaagatttaatattgattctgaaattattcaaaattcttcactctcaatgaaagaaattattcagttctttcaactttcaccatcatctttatcaaaaatcaataatatttcaattgaattatttgaatttgcatttaaatatctagaattaattgaaaaatcatgtacaaaacaacaaccaaactattcaaacagtataaaagatgcagcaaatgaaaaaatgggtgaattagtatctttatgtttatcaaattatccaaataatcaaaaatcatcattactttgggaaaaatggttatcaagaaatccaacctcacaattactatcacttttatcaaatttaaatgtaaaatcttcaactactataattaataataatattaataataataataataataataataataataataataataataataataataataataataataataataataataataataattcaattttaaattttatatctggcattaatagtaataaaataaatactccaaaatctaataataataaatttaaagaaaatggaattagaataatttgtttctcaaaagatagagcatttcaattaaaagaatatcttagaacattttttaaatatttaaaaaatgatgataatggaaatgataaatttgaaattattgttgatgtattatttacatattcaaatgagaaattcaaaaactcttatcaattagttattgaaagttttccacaagttaattttattaaagaagagaatttcactgatcaattaattaatttagttcaaaaaacaaataaacttgaatatgtcatgttttcagttgatgatattctttattataatgaattcaatctcaaagaatattgtttatctttgaatagtgagccattggcattaggtttctatatgaagttaaataaaaatattacctattgtcatacttgtaatcaagatataacaataccattaaattcaaatactattagtagaacagagaataattttaaatatttaaaatggaatagaaatgataatgattgtaaaaaggattggaattatccatgggatttatgttcaaccatttatagatgtaatgatattgattcaatcattaatggtatagttaaatattatggaattagaaatggtattaatcatccaaatagattcgaattcaatggtaatagaccaatcattcaaaagcaaatctatcaaaataaaccctactgtttatgtttatcagatcactattctccaatgtctgttgtaactattaatagagttcaagatgtctatgataatccaatttatgaccaaaccctatctttagatgatttagatcaattactttattcaaacaaatcattaaatgatgaaaaatataaagaaaatagtttatctttaaattttaaaagtgttcatattggtgaactttttatttcttaa

SEQ ID NO: 4 - protein, 329 aa, Dictyostellium discoideum
MSILNFISGINSNKINTPKSNNNKFKENGIRIICFSKDRAFQLKEYLRTFFKYLKNDDNGNDKFEIIVDVLFTYSNEKFKNSYQLVIESFPQVNFIKEENFTDQLINLVQKTNKLEYVMFSVDDILYYNEFNLKEYCLSLNSEPLALGFYMKLNKNITYCHTCNQDITIPLNSNTISRTENNFKYLKWNRNDNDCKKDWNYPWDLCSTIYRCNDIDSIINGIVKYYGIRNGINHPNRFEFNGNRPIIQKQIYQNKPYCLCLSDHYSPMSVVTINRVQDVYDNPIYDQTLSLDDLDQLLYSNKSLNDEKYKENSLSLNFKSVHIGELFIS

SEQ ID NO: 5 - DNA, 990 bp, Artificial sequence
  codon optimized sequence encoding part of SEQ ID NO 2
atgagcattctgaattttattagcggcattaatagcaataaaattaataccccgaaaagcaacaataacaaatttaaagagaatggcattcgcattatttgcttcagcaaagatcgtgcattccagctgaaagaatatctgcgcaccttcttcaaatatctgaaaaatgatgataatggcaatgataaatttgaaattattgtggatgtgctgtttacctatagcaatgaaaaattcaaaaatagctatcagctggtgatcgaaagctttccgcaggttaactttattaaagaagaaaactttaccgatcagctgattaacctggtgcagaaaaccaacaaactggaatatgtgatgttcagcgtggatgatatcctgtattacaacgagttcaatctgaaagagtattgcctgagcctgaatagcgaaccgctggcactgggtttttatatgaaactgaataaaaatattacctattgccatacctgcaaccaggatattaccattccgctgaatagcaataccattagccgcaccgaaaataactttaaatacctgaaatggaatcgcaacgataatgattgcaaaaaagactggaactatccgtgggatctgtgtagcaccatttatcgttgcaacgacattgacagcatcattaatggtattgtgaaatattatggtattcgcaacggcattaatcatccgaatcgctttgaatttaatggcaaccgtccgattattcagaaacaaatctaccagaacaaaccgtattgtctgtgcctgagcgatcattattcaccgatgagcgttgttaccattaatcgtgttcaggatgtgtatgataacccgatttatgatcagaccctgagcctggatgatctggatcaactgctgtatagcaataaatccctgaacgatgaaaaatataaagaaaacagcctgagtctgaacttcaaaagcgttcatattggcgaactgttcatcagctaa

SEQ ID NO: 6 - DNA, 987 bp, Dictyostellium discoideum
tcaattttaaattttatatctggcattaatagtaataaaataaatactccaaaatctaataataataaatttaaagaaaatggaattagaataatttgtttctcaaaagatagagcatttcaattaaaagaatatcttagaacattttttaaatatttaaaaaatgatgataatggaaatgataaatttgaaattattgttgatgtattatttacatattcaaatgagaaattcaaaaactcttatcaattagttattgaaagttttccacaagttaattttattaaagaagagaatttcactgatcaattaattaatttagttcaaaaaacaaataaacttgaatatgtcatgttttcagttgatgatattctttattataatgaattcaatctcaaagaatattgtttatctttgaatagtgagccattggcattaggtttctatatgaagttaaataaaaatattacctattgtcatacttgtaatcaagatataacaataccattaaattcaaatactattagtagaacagagaataattttaaatatttaaaatggaatagaaatgataatgattgtaaaaaggattggaattatccatgggatttatgttcaaccatttatagatgtaatgatattgattcaatcattaatggtatagttaaatattatggaattagaaatggtattaatcatccaaatagattcgaattcaatggtaatagaccaatcattcaaaagcaaatctatcaaaataaaccctactgtttatgtttatcagatcactattctccaatgtctgttgtaactattaatagagttcaagatgtctatgataatccaatttatgaccaaaccctatctttagatgatttagatcaattactttattcaaacaaatcattaaatgatgaaaaatataaagaaaatagtttatctttaaattttaaaagtgttcatattggtgaactttttatttcttaa

SEQ ID NO: 7 - DNA, 74 bp, Artificial sequence
  Primer
cataatggatttccttacgcgaaatacgggcagacatggcctgcccggttattagtgtaggctggagctgcttc

SEQ ID NO: 8 - DNA, 71 bp, Artificial sequence
  Primer
gtatgttgtgtggaattgtgagcggataacaatttcacacaggaaacagctcatatgaatatcctccttag

SEQ ID NO: 9 - DNA, 75 bp, Artificial sequence
  Primer
agaccgccggttttaagcagcgggaacatctctgaacatacatgtaaaacctgcagtgtaggctggagctgcttc

SEQ ID NO: 10 - DNA, 82 bp, Artificial sequence
  Primer
gtctggcagggacctgcacacggattgtgtgtgttccagagatgataaaaaaggagttagtccatatgaatatcctccttag

SEQ ID NO: 11 - DNA, 70 bp, Artificial sequence
  Primer
catatttctgtcacactctttagtgattgataacaaaagaggtgccaggagtgtaggctggagctgcttc

SEQ ID NO: 12 - DNA, 70 bp, Artificial sequence
  Primer
taaaaacgtttaaccagcgactcccccgcttctcgcgggggagttttctgcatatgaatatcctccttag

SEQ ID NO: 13 - DNA, 70 bp, Artificial sequence
  Primer
ggcgctacaatcttccaaagtcacaattctcaaaatcagaagagtattgcgtgtaggctggagctgcttc

SEQ ID NO: 14 - DNA, 70 bp, Artificial sequence
  Primer
ggttgccggatgcggcgtgaacgccttatccggcctacatatcgacgatgcatatgaatatcctccttag

SEQ ID NO: 15 - DNA, 69 bp, Artificial sequence
  Primer
gacttccggcaacagatttcattttgcattccaaagttcagaggtagtcgtgtaggctggagctgcttc

SEQ ID NO: 16 - DNA, 69 bp, Artificial sequence
  Primer
gcttctgtcatcggtttcagggtaaaggaatctgcctttttccgaaatccatatgaatatcctccttag

SEQ ID NO: 17 - DNA, 71 bp, Artificial sequence
  Primer
cactttccgctgattcggtgccagactgaaatcagcctataggaggaaatggtgtaggctggagctgcttc

SEQ ID NO: 18 - DNA, 70 bp, Artificial sequence
  Primer
gttgccgacaggttggtgatgattcccccaatgctgggggaatgtttttgcatatgaatatcctccttag

SEQ ID NO: 19 - DNA, 70 bp, Artificial sequence
  Primer
tgagaaggtttgcggaactatctaaaacgttgcagacaaaggacaaagcagtgtaggctggagctgcttc

SEQ ID NO: 20 - DNA, 71 bp, Artificial sequence
  Primer
catacgtaaaaaagggcgatcttgcgaccgccctttttttattaaatgtgtcatatgaatatcctccttag

SEQ ID NO: 21 - DNA, 70 bp, Artificial sequence
  Primer
tgagaaggtttgcggaactatctaaaacgttgcagacaaaggacaaagcaacgaaaggctcagtcgaaag

SEQ ID NO: 22 - DNA, 71 bp, Artificial sequence
  Primer
catacgtaaaaaagggcgatcttgcgaccgccctttttttattaaatgtgtagaactccagcatgagatcc

SEQ ID NO: 23 - DNA, 70 bp, Artificial sequence; identical to SEQ ID NO: 19
  Primer

SEQ ID NO: 24 - DNA, 71 bp, Artificial sequence
  Primer
catacgtaaaaaagggcgatcttgcgaccgccctttttttattaaatgtgtcatccgtcaggatggccttc

SEQ ID NO: 25 - DNA, 72 bp, Artificial sequence
  Primer
gccacgcgtgagaacgtaaaaaaagcacccatactcaggagcactctcaattgtgtaggctggagctgcttc

SEQ ID NO: 26 - DNA, 75 bp, Artificial sequence
  Primer
cacctgtaaaaaaggcagccatctggctgccttagtctccccaacgtcttacggacatatgaatatcctccttag

SEQ ID NO: 27 - DNA, 70 bp, Artificial sequence
  Primer
cgagaaggcccggattgtcatggacgatgagatacaccggaatatcatgggtgtaggctggagctgcttc

SEQ ID NO: 28 - DNA, 76 bp, Artificial sequence
  Primer
ccaggtatttacagtgtgagaaagaattattttgactttagcggagcagttgaagacatatgaatatcctccttag

SEQ ID NO: 29 - DNA, 70 bp, Artificial sequence
  Primer
atatccagccagtcttccggctgtagtcctaacagagcactgttactgtcagcattacacgtcttgagcg

SEQ ID NO: 30 - DNA, 70 bp, Artificial sequence
  Primer
gctttaagtggttgagatcacatttccttgctcatccccgcaactcctcccatatgaatatcctccttag

SEQ ID NO: 31 - DNA, 68 bp, Artificial sequence
  Primer
atatccagccagtcttccggctgtagtcctaacagagcactgttactgtcgtaaaacgacggccagtg

SEQ ID NO: 32 - DNA, 72 bp, Artificial sequence
  Primer
caacggccattttttgcacttagatacagattttctgcgctgtattgcattgccgggatccgatgcatatgg

SEQ ID NO: 33 - DNA, 75 bp, Artificial sequence
  Primer
ttttattttgcccttcaatgggaccgctaccaaacatcaggaggatgaatgaaacagcattacacgtcttgagcg

SEQ ID NO: 34 - DNA, 70 bp, Artificial sequence
  Primer
ttccgttgaaggcaacagtaattgcgccccggttaagcccgcgccgatcccatatgaatatcctccttag

SEQ ID NO: 35 - DNA, 71 bp, Artificial sequence
  Primer
gtagcattgttcctaagtatgactccatttttccaggaatggtcgcaaatcgtgtaggctggagctgcttc

SEQ ID NO: 36 - DNA, 70 bp, Artificial sequence
  Primer
ttcacgccgcatccggcaagcaaaccagctcataagccgggagaacaacccatatgaatatcctccttag

SEQ ID NO: 37 - DNA, 70 bp, Artificial sequence
  Primer
ttcacgccgcatccggcaagcaaaccagctcataagccgggagaacaaccccgcttacagacaagctgtg

SEQ ID NO: 38 - DNA, 71 bp, Artificial sequence
  Primer
gtagcattgttcctaagtatgactccatttttccaggaatggtcgcaaatcagccatgacccgggaattac

SEQ ID NO: 39 - DNA, 70 bp, Artificial sequence
  Primer
atcgccgaccacttcgcgccgctgatggttttttcacgtaagctcatatcccgcttacagacaagctgtg

SEQ ID NO: 40 - DNA, 70 bp, Artificial sequence
  Primer
ggatcttcccttaccccactgcgggtaaggggctaataacaggaacaacgagccatgacccgggaattac

SEQ ID NO: 41 - DNA, 42 bp, Artificial sequence
  Primer
gggggcccccgggggtatgagcttacgtgaaaaaaccatcag

SEQ ID NO: 42 - DNA, 43 bp, Artificial sequence
  Primer
gggcccgggcccgggcgttgttcctgttattagccccttaccc

SEQ ID NO: 43 - DNA, 70 bp, Artificial sequence
  Primer
atcgccgaccacttcgcgccgctgatggttttttcacgtaagctcatatcgtgtaggctggagctgcttc

SEQ ID NO: 44 - DNA, 70 bp, Artificial sequence
  Primer
ggatcttcccttaccccactgcgggtaaggggctaataacaggaacaacgcatatgaatatcctccttag

SEQ ID NO: 45 - DNA, 70 bp, Artificial sequence
  Primer
ttttgatatcgaaccagacgctccattcgcggatgtactcaaggtcgaacgtgtaggctggagctgcttc

SEQ ID NO: 46 - DNA, 70 bp, Artificial sequence
  Primer
tctatggtgcaacgcttttcagatatcaccatcatgtttgccggactatgcatatgaatatcctccttag

SEQ ID NO: 47 - DNA, 70 bp, Artificial sequence
  Primer
tagccaaatgcgttggcaaacagagattgtgttttttctttcagactcatctttgtttcctccgaattcg

SEQ ID NO: 48 - DNA, 70 bp, Artificial sequence
  Primer
cggttcgacgcatgcaggcatgaaaccgcgtcttttttcagataaaaagccatatgaatatcctccttag

SEQ ID NO: 49 - DNA, 70 bp, Artificial sequence
  Primer
accaatcaaattcacgcggccaggcgcctgaatggtgtgagtggcagggtagccaaatgcgttggcaaac

SEQ ID NO: 50 - DNA, 70 bp, Artificial sequence
  Primer
gtcggtagtgctgaccttgccggaggcggccttagcaccctctccggccaacggttcgacgcatgcaggc

SEQ ID NO: 51 - DNA, 1841 bp, Escherichia coli
agcatgatcgaacacatcatgcagtcgatgcaattcccggcggaattgattgagaaggtttgcggaactatctaaaacgttgcagacaaaggacaaagcaatggcaatccacaatcgtgcaggccaacctgcacaacagagtgatttgattaacgtcgcccaactgacggcgcaatattatgtactgaaaccagaagcagggaatgcggagcacgcggtgaaattcggtacttccggtcaccgtggcagtgcagcgcgccacagctttaacgagccgcacattctggcgatcgctcaggcaattgctgaagaacgtgcgaaaaacggcatcactggcccttgctatgtgggtaaagatactcacgccctgtccgaacctgcattcatttccgttctggaagtgctggcagcgaacggcgttgatgtcattgtgcaggaaaacaatggcttcaccccgacgcctgccgtttccaatgccatcctggttcacaataaaaaaggtggcccgctggcagacggtatcgtgattacaccgtcccataacccgccggaagatggtggaatcaaatacaatccgccaaatggtggcccggctgataccaacgtcactaaagtggtggaagacagggccaacgcactgctggccgatggcctgaaaggcgtgaagcgtatctccctcgacgaagcgatggcatccggtcatgtgaaagagcaggatctggtgcagccgttcgtggaaggtctggccgatatcgttgatatggccgcgattcagaaagcgggcctgacgctgggcgttgatccgctgggcggttccggtatcgaatactggaagcgtattggcgagtattacaacctcaacctgactatcgttaacgatcaggtcgatcaaaccttccgctttatgcaccttgataaagacggcgcgatccgtatggactgctcctccgagtgtgcgatggcgggcctgctggcactgcgtgataagttcgatctggcgtttgctaacgacccggattatgaccgtcacggtatcgtcactccggcaggtttgatgaatccgaaccactacctggcggtggcaatcaattacctgttccagcatcgtccgcagtggggcaaagatgttgccgtcggtaaaacgctggtttcatctgcgatgatcgaccgtgtggtcaacgacttgggccgtaaactggtagaagtcccggtaggtttcaaatggtttgtcgatggtctgttcgacggcagcttcggctttggcggcgaagagagtgcaggggcttccttcctgcgtttcgacggcacgccgtggtccaccgacaaagacggcatcatcatgtgtctgctggcggcggaaatcaccgctgtcaccggtaagaacccgcaggaacactacaacgaactggcaaaacgctttggtgcgccgagctacaaccgtttgcaggcagctgcgacttccgcacaaaaagcggcgctgtctaagctgtctccggaaatggtgagcgccagcaccctggcaggtgacccgatcaccgcgcgcctgactgctgctccgggcaacggtgcttctattggcggtctgaaagtgatgactgacaacggctggttcgccgcgcgtccgtcaggcacggaagacgcatataagatctactgcgaaagcttcctcggtgaagaacatcgcaagcagattgagaaagaagcggttgagattgttagcgaagttctgaaaaacgcgtaaacacatttaataaaaaaagggcggtcgcaagatcgcccttttttacgtatgacaaacacagaattgcctgatgcgctacgcttatcaggcctacgaggat

SEQ ID NO: 52 - DNA, 509 bp, Escherichia coli
cgtacacgcgtttactttgcggcagatgaacaaacgctgctgaaaaatggtaatcagaccaagccgaaacatgtgccaggcacgccgtattgggtgatcaccaacaccaacaccggccgtaaatgcagcatgatcgaacacatcatgcagtcgatgcaattcccggcggaattgattgagaaggtttgcggaactatctaaaacgttgcagacaaaggacaaagcagtgtaggctggagctgcttcgaagttcctatactttctagagaataggaacttcggaataggaactaaggaggatattcatatgacacatttaataaaaaaagggcggtcgcaagatcgcccttttttacgtatgacaaacacagaattgcctgatgcgctacgcttatcaggcctacgaggatggtgcaatatattgaatttaagcgattttgtaggccggataaggcgttcacgccgcatccggcaaaaacaacgaacactttgtcaacaaactgagtagc

SEQ ID NO: 53 - DNA, 2061 bp, Escherichia coli
  misc_feature (707)..(707): n is a, c, g, or t
cgtacacgcgtttactttgcggcagatgaacaaacgctgctgaaaaatggtaatcagaccaagccgaaacatgtgccaggcacgccgtattgggtgatcaccaacaccaacaccggccgtaaatgcagcatgatcgaacacatcatgcagtcgatgcaattcccggcggaattgattgagaaggtttgcggaactatctaaaacgttgcagacaaaggacaaagcagtgtaggctggagctgcttcgaagttcctatactttctagagaataggaacttcggaataggaactaaggaggatattcatatggaccgatatcccgggcggccgcttcatttataaatttcttgacattttggaatagatgtgatataatgtgtacatatccatggcggccgctctagaagaagcttgggatccgtcgacctcgaattcggaggaaacaaagatggggggttctcatcatcatcatcatcatggtatggctagcatgagtaaaggagaagaacttttcactggagttgtcccaattcttgttgaattagatggtgatgttaatgggcacaaattttctgtcagtggagagggtgaaggtgatgcaacatacggaaaacttacccttaaatttatttgcactactggaaaactacctgttccatggccaacacttgtcactactttcgggtatggtgttcaatgctttgcnagatacccagatcatatgaaacagcatgactttttcaagagtgccatgcccgaaggttatgtacaggaaagaactatatttttcaaagatgacgggaactacaagacacgtgctgaagtcaagtttgaaggtgatacccttgttaatagaatcgagttaaaaggtattgattttaaagaagatggaaacattcttggacacaaattggaatacaactataactcacacaatgtatacatcatggcagacaaacaaaagaatggaatcaaagttaacttcaaaattagacacaacattgaagatggaagcgttcaactagcagaccattatcaacaaaatactccaattggcgatggccctgtccttttaccagacaaccattacctgtccacacaatctgccctttcgaaagatcccaacgaaaagagagaccacatggtccttcttgagtttgtaacagctgctgggattacacatggcatggatgaactatacaaataactgcaggtcgaccatatgggagagctcccaacgcgttggatgcaggcatgcaagcttggctgttttggcggatgagagaagattttcagcctgatacagattaaatcagaacgcagaagcggtctgataaaacagaatttgcctggcggcagtagcgcggtggtcccacctgaccccatgccgaactcagaagtgaaacgccgtagcgccgatggtagtgtggggtctccccatgcgagagtagggaactgccaggcatcaaataaaacgaaaggctcagtcgaaagactgggcctttcgttttatctgttgtttgtcggtgaacgctctcctgagtaggacaaatccgccgggagcggatttgaacgttgcgaagcaacggcccggagggtggcgggcaggacgcccgccataaactgccaggcatcaaattaagcagaaggccatcctgacggatgctactgcgaaagcttcctcggtgaagaacatcgcaagcagattgagaaagaagcggttgagattgttagcgaagttctgaaaaacgcgtaactactgcgaaagcttcctcggtgaagaacatcgcaagcagattgagaaagaagcggttgagattgttagcgaagttctgaaaaacgcgtaaacacatttaataaaaaaagggcggtcgcaagatcgcccttttttacgtatgacaaacacagaattgcctgatgcgctacgcttatcaggcctacgaggatggtgcaatatattgaatttaagcgattttgtaggccggataaggcgttcacgccgcatccggcaaaaacaacgaacactttgtcaacaaactgagtagctcaaggaaatccca

SEQ ID NO: 54 - DNA, 1735 bp, Escherichia coli
cgtacacgcgtttactttgcggcagatgaacaaacgctgctgaaaaatggtaatcagaccaagccgaaacatgtgccaggcacgccgtattgggtgatcaccaacaccaacaccggccgtaaatgcagcatgatcgaacacatcatgcagtcgatgcaattcccggcggaattgattgagaaggtttgcggaactatctaaaacgttgcagacaaaggacaaagcaacgaaaggctcagtcgaaagactgggcctttcgttttatctgttgtttgtcggtgaacgctctcctgagtaggacaaatccgccgggagcggatttgaacgttgcgaagcaacggcccggagggtggcgggcaggacgcccgccataaactgccaggcatcaaattaagcagaaggccatcctgacggatggcctttttgcgtggccagtgccaagcttgcatgcagattgcagcattacacgtcttgagcgattgtgtaggctggagctgcttcgaagttcctatactttctagagaataggaacttcggaataggaacttcaagatcccctcacgctgccgcaagcactcagggcgcaagggctgctaaaggaagcggaacacgtagaaagccagtccgcagaaacggtgctgaccccggatgaatgtcagctactgggctatctggacaagggaaaacgcaagcgcaaagagaaagcaggtagcttgcagtgggcttacatggcgatagctagactgggcggttttatggacagcaagcgaaccggaattgccagctggggcgccctctggtaaggttgggaagccctgcaaagtaaactggatggctttcttgccgccaaggatctgatggcgcaggggatcaagatctgatcaagagacaggatgaggatcgtttcgcaagatcccctcacgctgccgcaagcactcagggcgcaagggctgctaaaggaagcggaacacgtagaaagccagtccgcagaaacggtgctgaccccggatgaatgtcagctactgggctatctggacaagggaaaacgcaagcgcaaagagaaagcaggtagcttgcagtgggcttacatggcgatagctagactgggcggttttatggacagcaagcgaaccggaattgccagctggggcgccctctggtaaggttgggaagccctgcaaagtaaactggatggctttcttgccgccaaggatctgatggcgcaggggatcaagatctgatcaagagacaggatgaggatcgtttcgcgcgggactctggggttcgaaatgaccgaccaagcgacgcccaacctgccatcacgagatttcgattccaccgccgccttctatgaaaggttgggcttcggaatcgttttccgggacgccggctggatgatcctccagcgcggggatctcatgctggagttctctactgcgaaagcttcctcggtgaagaacatcgcaagcagattgagaaagaagcggttgagattgttagcgaagttctgaaaaacgcgtaaacacatttaataaaaaaagggcggtcgcaagatcgcccttttttacgtatgacaaacacagaattgcctgatgcgctacgcttatcaggcctacgaggatggtgcaatatattgaatttaagcgattttgtaggccggataaggcgttcacgccgcatccggcaaaaacaacgaacactttgtcaacaaactgagtagctcaaggaaatccca